European Patent Application EP 4 775 592 A2, published July 15, 2026. Title: FGF21 compound / GLP-1R agonist combinations with optimized activity ratio. Applicant: SANOFI. Application EP. The sequence listing filed with the application follows.

SEQUENCE LISTING (70 sequences)

SEQ ID NO: 1 - protein, 209 aa, Homo sapiens [sequence omitted]

SEQ ID NO: 2 - protein, 181 aa, Homo sapiens
HPIPDSSPLLQFGGQVRQRYLYTDDAQQTEAHLEIREDGTVGGAADQSPESLLQLKALKPGVIQILGVKTSRFLCQRPDGALYGSLHFDPEACSFRELLLEDGYNVYQSEAHGLPLHLPGNKSPHRDPAPRGPARFLPLPGLPPAPPEPPGILAPQPPDVGSSDPLSMVGPSQGRSPSYAS

SEQ ID NO: 3 - protein, 181 aa, synthetic construct
  REGION 1..181: note = FGF21(His29-Ser209) A59C,G71C
HPIPDSSPLLQFGGQVRQRYLYTDDAQQTECHLEIREDGTVGCAADQSPESLLQLKALKPGVIQILGVKTSRFLCQRPDGALYGSLHFDPEACSFRELLLEDGYNVYQSEAHGLPLHLPGNKSPHRDPAPRGPARFLPLPGLPPAPPEPPGILAPQPPDVGSSDPLSMVGPSQGRSPSYAS

SEQ ID NO: 4 - protein, 181 aa, synthetic construct
  REGION 1..181: note = FGF21(His29-Ser209) Q55C,N149C,G198Y
HPIPDSSPLLQFGGQVRQRYLYTDDACQTEAHLEIREDGTVGGAADQSPESLLQLKALKPGVIQILGVKTSRFLCQRPDGALYGSLHFDPEACSFRELLLEDGYNVYQSEAHGLPLHLPGCKSPHRDPAPRGPARFLPLPGLPPAPPEPPGILAPQPPDVGSSDPLSMVYPSQGRSPSYAS

SEQ ID NO: 5 - protein, 180 aa, synthetic construct
  REGION 1..180: note = FGF21(His29-Ser209) Q55C,P147C,delP199
HPIPDSSPLLQFGGQVRQRYLYTDDACQTEAHLEIREDGTVGGAADQSPESLLQLKALKPGVIQILGVKTSRFLCQRPDGALYGSLHFDPEACSFRELLLEDGYNVYQSEAHGLPLHLCGNKSPHRDPAPRGPARFLPLPGLPPAPPEPPGILAPQPPDVGSSDPLSMVGSQGRSPSYAS

SEQ ID NO: 6 - protein, 180 aa, synthetic construct
  REGION 1..180: note = FGF21(His29-Ser209) Q55C,N149C,delP199
HPIPDSSPLLQFGGQVRQRYLYTDDACQTEAHLEIREDGTVGGAADQSPESLLQLKALKPGVIQILGVKTSRFLCQRPDGALYGSLHFDPEACSFRELLLEDGYNVYQSEAHGLPLHLPGCKSPHRDPAPRGPARFLPLPGLPPAPPEPPGILAPQPPDVGSSDPLSMVGSQGRSPSYAS

SEQ ID NO: 7 - protein, 30 aa, Homo sapiens
HAEGTFTSDVSSYLEGQAAKEFIAWLVKGR

SEQ ID NO: 8 - protein, 39 aa, synthetic construct
  REGION 1..39: note = GLP1(7-36) A8G,V16L,S18K,Y19Q,L20M,G22E,Q23E,A25V,K26R,E27L,A30E,V33K,K34N,R 36G,insPSSGAPPPS
HGEGTFTSDLSKQMEEEAVRLFIEWLKNGGPSSGAPPPS

SEQ ID NO: 9 - protein, 39 aa, synthetic construct
  REGION 1..39: note = GLP1(7-36) A8G,V16L,S18K,Y19Q,G22E,Q23E,A25V,K26Q,E27L,A30E,V33L,K34A,G35T,R 36G,insPSSGAPPPS
HGEGTFTSDLSKQLEEEAVQLFIEWLLATGPSSGAPPPS

SEQ ID NO: 10 - protein, 39 aa, synthetic construct
  REGION 1..39: note = GLP1(7-36) A8G,V16L,S18I,Y19Q,E21D,G22E,Q23E,A25V,K26R,E27L,A30E,V33L,K34A,G 35T,R36G,insPVSGAPPPS
HGEGTFTSDLSIQLDEEAVRLFIEWLLATGPVSGAPPPS

SEQ ID NO: 11 - protein, 39 aa, synthetic construct
  REGION 1..39: note = GLP1(7-36) A8G,V16L,S18I,Y19Q,E21D,G22E,Q23E,A25V,K26R,E27L,A30E,V33E,K34A,G 35T,R36G,insPVSGAPPPS
HGEGTFTSDLSIQLDEEAVRLFIEWLEATGPVSGAPPPS

SEQ ID NO: 12 - protein, 40 aa, synthetic construct
  REGION 1..40: note = GLP1(7-36) insG,A8G,V16L,S18I,Y19Q,G22E,Q23E,A25V,K26R,E27L,A30E,V33L,K34A,R 36G,insPSSGAPPPS
GHGEGTFTSDLSIQLEEEAVRLFIEWLLAGGPSSGAPPPS

SEQ ID NO: 13 - protein, 40 aa, synthetic construct
  REGION 1..40: note = GLP1(7-36) insG,A8G,V16L,S18I,Y19Q,G22E,Q23E,A25V,K26R,E27L,A30E,V33L,K34A,G 35T,R36G,insPSSGAPPPS
GHGEGTFTSDLSIQLEEEAVRLFIEWLLATGPSSGAPPPS

SEQ ID NO: 14 - protein, 40 aa, synthetic construct
  REGION 1..40: note = GLP1(7-36) A8G,V16L,S18K,Y19Q,E21D,G22E,Q23E,A25V,K26Q,E27L,A30E,V33L,K34A,G 35T,R36G,insPSSGEPPPES
HGEGTFTSDLSKQLEEEAVQLFIEWLLATGPSSGEPPPES

SEQ ID NO: 15 - protein, 30 aa, synthetic construct
  REGION 1..30: note = GLP1(7-36) A8G,V16L,S18K,Y19Q,L20M,E21D,G22E,Q23E,A25V,K26R,E27L,A30E,V33K,K 34N,R36G
HGEGTFTSDLSKQMEEEAVRLFIEWLKNGG

SEQ ID NO: 16 - protein, 30 aa, synthetic construct
  REGION 1..30: note = GLP1(7-36) A8G,V16L,S18K,Y19Q,G22E,Q23E,A25V,K26Q,E27L,A30E,V33L,K34A,G35T,R 36G
HGEGTFTSDLSKQLEEEAVQLFIEWLLATG

SEQ ID NO: 17 - protein, 39 aa, synthetic construct
  REGION 1..39: note = GLP1(7-36) A8G,V16L,S18K,Y19Q,G22E,Q23E,A25V,K26Q,E27L,A30E,V33L,K34A,G35T,R 36G,insPSSGEPPPE
HGEGTFTSDLSKQLEEEAVQLFIEWLLATGPSSGEPPPE

SEQ ID NO: 18 - protein, 40 aa, synthetic construct
  REGION 1..40: note = GLP1(7-36) insG,A8G,V16L,S18K,Y19Q,G22E,Q23E,A24R,A25V,K26Q,A30E,insPSSGAPPP S
GHGEGTFTSDLSKQLEEERVQEFIEWLVKGRPSSGAPPPS

SEQ ID NO: 19 - protein, 39 aa, synthetic construct
  REGION 1..39: note = GLP1(7-36) A8G,V16L,S18K,Y19Q,G22E,Q23E,A25V,K26Q,E27L,A30E,V33E,K34A,G35T,R 36G,insPSSGAPPPS
HGEGTFTSDLSKQLEEEAVQLFIEWLEATGPSSGAPPPS

SEQ ID NO: 20 - protein, 38 aa, synthetic construct
  REGION 1..38: note = GLP1(7-36) insG,A8G,V16L,S18I,Y19Q,G22E,Q23E,A25V,K26R,E27L,A30E,V33L,K34A,R 36G,insPKKQRLS
GHGEGTFTSDLSIQLEEEAVRLFIEWLLAGGPKKQRLS

SEQ ID NO: 21 - protein, 228 aa, synthetic construct
  REGION 1..228: note = IgG4 Fc variant, IGHG4_HUMAN (Glu99-Gly326)
ESKYGPPCPPCPAPEFEGGPSVFLFPPKPKDTLMISRTPEVTCVVVDVSQEDPEVQFNWYVDGVEVHNAKTKPREEQFNSTYRVVSVLTVLHQDWLNGKEYKCKVSNKGLPSSIEKTISKAKGQPREPQVYTLPPSQEEMTKNQVSLTCLVKGFYPSDIAVEWESNGQPENNYKTTPPVLDSDGSFFLYSRLTVDKSRWQEGNVFSCSVMHEALHNHYTQKSLSLSLG

SEQ ID NO: 22 - protein, 19 aa, synthetic construct
  REGION 1..19: note = (G7S)(G4S)(G4S)A Linker (19GS)
GGGGGGGSGGGGSGGGGSA

SEQ ID NO: 23 - protein, 7 aa, synthetic construct
  REGION 1..7: note = (G3S)(GS)A Linker (7GS)
GGGSGSA

SEQ ID NO: 24 - protein, 474 aa, synthetic construct
  REGION 1..474: note = GLP1(7-36) A8G,V16L,S18K,Y19Q,L20M,G22E,Q23E,A25V,K26R,E27L,A30E,V33K,K34N,R 36G,insPSSGAPPPS_[19GS]_IgG4 Fc_variant [7GS]_ FGF21(His29-Ser209)_A59C,G71C
HGEGTFTSDLSKQMEEEAVRLFIEWLKNGGPSSGAPPPSGGGGGGGSGGGGSGGGGSAESKYGPPCPPCPAPEFEGGPSVFLFPPKPKDTLMISRTPEVTCVVVDVSQEDPEVQFNWYVDGVEVHNAKTKPREEQFNSTYRVVSVLTVLHQDWLNGKEYKCKVSNKGLPSSIEKTISKAKGQPREPQVYTLPPSQEEMTKNQVSLTCLVKGFYPSDIAVEWESNGQPENNYKTTPPVLDSDGSFFLYSRLTVDKSRWQEGNVFSCSVMHEALHNHYTQKSLSLSLGGGGSGSAHPIPDSSPLLQFGGQVRQRYLYTDDAQQTECHLEIREDGTVGCAADQSPESLLQLKALKPGVIQILGVKTSRFLCQRPDGALYGSLHFDPEACSFRELLLEDGYNVYQSEAHGLPLHLPGNKSPHRDPAPRGPARFLPLPGLPPAPPEPPGILAPQPPDVGSSDPLSMVGPSQGRSPSYAS

SEQ ID NO: 25 - protein, 474 aa, synthetic construct
  REGION 1..474: note = GLP1(7-36) A8G,V16L,S18K,Y19Q,G22E,Q23E,A25V,K26Q,E27L,A30E,V33L,K34A,G35T,R 36G,insPSSGAPPPS_[19GS] _IgG4 Fc variant_[7GS]_FGF21(His29-Ser209)Q55C,N149C,G198Y
HGEGTFTSDLSKQLEEEAVQLFIEWLLATGPSSGAPPPSGGGGGGGSGGGGSGGGGSAESKYGPPCPPCPAPEFEGGPSVFLFPPKPKDTLMISRTPEVTCVVVDVSQEDPEVQFNWYVDGVEVHNAKTKPREEQFNSTYRVVSVLTVLHQDWLNGKEYKCKVSNKGLPSSIEKTISKAKGQPREPQVYTLPPSQEEMTKNQVSLTCLVKGFYPSDIAVEWESNGQPENNYKTTPPVLDSDGSFFLYSRLTVDKSRWQEGNVFSCSVMHEALHNHYTQKSLSLSLGGGGSGSAHPIPDSSPLLQFGGQVRQRYLYTDDACQTEAHLEIREDGTVGGAADQSPESLLQLKALKPGVIQILGVKTSRFLCQRPDGALYGSLHFDPEACSFRELLLEDGYNVYQSEAHGLPLHLPGCKSPHRDPAPRGPARFLPLPGLPPAPPEPPGILAPQPPDVGSSDPLSMVYPSQGRSPSYAS

SEQ ID NO: 26 - protein, 473 aa, synthetic construct
  REGION 1..473: note = GLP1(7-36) A8G,V16L,S18I,Y19Q,E21D,G22E,Q23E,A25V,K26R,E27L,A30E,V33L,K34A,G 35T,R36G,insPVSGAPPPS_[19GS]_IgG4 Fc_variant [7GS]_FGF21(His29-Ser209)Q55C,P147C,delP199
HGEGTFTSDLSIQLDEEAVRLFIEWLLATGPVSGAPPPSGGGGGGGSGGGGSGGGGSAESKYGPPCPPCPAPEFEGGPSVFLFPPKPKDTLMISRTPEVTCVVVDVSQEDPEVQFNWYVDGVEVHNAKTKPREEQFNSTYRVVSVLTVLHQDWLNGKEYKCKVSNKGLPSSIEKTISKAKGQPREPQVYTLPPSQEEMTKNQVSLTCLVKGFYPSDIAVEWESNGQPENNYKTTPPVLDSDGSFFLYSRLTVDKSRWQEGNVFSCSVMHEALHNHYTQKSLSLSLGGGGSGSAHPIPDSSPLLQFGGQVRQRYLYTDDACQTEAHLEIREDGTVGGAADQSPESLLQLKALKPGVIQILGVKTSRFLCQRPDGALYGSLHFDPEACSFRELLLEDGYNVYQSEAHGLPLHLCGNKSPHRDPAPRGPARFLPLPGLPPAPPEPPGILAPQPPDVGSSDPLSMVGSQGRSPSYAS

SEQ ID NO: 27 - protein, 473 aa, synthetic construct
  REGION 1..473: note = GLP1(7-36) A8G,V16L,S18I,Y19Q,E21D,G22E,Q23E,A25V,K26R,E27L,A30E,V33E,K34A,G 35T,R36G,insPVSGAPPPS_[19GS]_IgG4 Fc_variant [7GS]_FGF21(His29-Ser209)Q55C,N149C,delP199
HGEGTFTSDLSIQLDEEAVRLFIEWLEATGPVSGAPPPSGGGGGGGSGGGGSGGGGSAESKYGPPCPPCPAPEFEGGPSVFLFPPKPKDTLMISRTPEVTCVVVDVSQEDPEVQFNWYVDGVEVHNAKTKPREEQFNSTYRVVSVLTVLHQDWLNGKEYKCKVSNKGLPSSIEKTISKAKGQPREPQVYTLPPSQEEMTKNQVSLTCLVKGFYPSDIAVEWESNGQPENNYKTTPPVLDSDGSFFLYSRLTVDKSRWQEGNVFSCSVMHEALHNHYTQKSLSLSLGGGGSGSAHPIPDSSPLLQFGGQVRQRYLYTDDACQTEAHLEIREDGTVGGAADQSPESLLQLKALKPGVIQILGVKTSRFLCQRPDGALYGSLHFDPEACSFRELLLEDGYNVYQSEAHGLPLHLPGCKSPHRDPAPRGPARFLPLPGLPPAPPEPPGILAPQPPDVGSSDPLSMVGSQGRSPSYAS

SEQ ID NO: 28 - protein, 474 aa, synthetic construct
  REGION 1..474: note = GLP1(7-36) insG,A8G,V16L,S18I,Y19Q,G22E,Q23E,A25V,K26R,E27L,A30E,V33L,K34A,R 36G,insPSSGAPPPS_[19GS] _IgG4 Fc_variant [7GS]_FGF21(His29-Ser209)Q55C,N149C,delP199
GHGEGTFTSDLSIQLEEEAVRLFIEWLLAGGPSSGAPPPSGGGGGGGSGGGGSGGGGSAESKYGPPCPPCPAPEFEGGPSVFLFPPKPKDTLMISRTPEVTCVVVDVSQEDPEVQFNWYVDGVEVHNAKTKPREEQFNSTYRVVSVLTVLHQDWLNGKEYKCKVSNKGLPSSIEKTISKAKGQPREPQVYTLPPSQEEMTKNQVSLTCLVKGFYPSDIAVEWESNGQPENNYKTTPPVLDSDGSFFLYSRLTVDKSRWQEGNVFSCSVMHEALHNHYTQKSLSLSLGGGGSGSAHPIPDSSPLLQFGGQVRQRYLYTDDACQTEAHLEIREDGTVGGAADQSPESLLQLKALKPGVIQILGVKTSRFLCQRPDGALYGSLHFDPEACSFRELLLEDGYNVYQSEAHGLPLHLPGCKSPHRDPAPRGPARFLPLPGLPPAPPEPPGILAPQPPDVGSSDPLSMVGSQGRSPSYAS

SEQ ID NO: 29 - protein, 474 aa, synthetic construct
  REGION 1..474: note = GLP1(7-36) insG,A8G,V16L,S18I,Y19Q,G22E,Q23E,A25V,K26R,E27L,A30E,V33L,K34A,G 35T,R36G,insPSSGAPPPS_[19GS]_Ig4G Fc_variant [7GS]_FGF21(His29-Ser209)Q55C,P147C,delP199
GHGEGTFTSDLSIQLEEEAVRLFIEWLLATGPSSGAPPPSGGGGGGGSGGGGSGGGGSAESKYGPPCPPCPAPEFEGGPSVFLFPPKPKDTLMISRTPEVTCVVVDVSQEDPEVQFNWYVDGVEVHNAKTKPREEQFNSTYRVVSVLTVLHQDWLNGKEYKCKVSNKGLPSSIEKTISKAKGQPREPQVYTLPPSQEEMTKNQVSLTCLVKGFYPSDIAVEWESNGQPENNYKTTPPVLDSDGSFFLYSRLTVDKSRWQEGNVFSCSVMHEALHNHYTQKSLSLSLGGGGSGSAHPIPDSSPLLQFGGQVRQRYLYTDDACQTEAHLEIREDGTVGGAADQSPESLLQLKALKPGVIQILGVKTSRFLCQRPDGALYGSLHFDPEACSFRELLLEDGYNVYQSEAHGLPLHLCGNKSPHRDPAPRGPARFLPLPGLPPAPPEPPGILAPQPPDVGSSDPLSMVGSQGRSPSYAS

SEQ ID NO: 30 - protein, 475 aa, synthetic construct
  REGION 1..475: note = GLP1(7-36) A8G,V16L,S18K,Y19Q,E21D,G22E,Q23E,A25V,K26Q,E27L,A30E,V33L,K34A,G 35T,R36G,insPSSGEPPPES_[19GS]_IgG4 Fc_variant [7GS]_FGF21(His29-Ser209)Q55C,N149C,G198Y
HGEGTFTSDLSKQLEEEAVQLFIEWLLATGPSSGEPPPESGGGGGGGSGGGGSGGGGSAESKYGPPCPPCPAPEFEGGPSVFLFPPKPKDTLMISRTPEVTCVVVDVSQEDPEVQFNWYVDGVEVHNAKTKPREEQFNSTYRVVSVLTVLHQDWLNGKEYKCKVSNKGLPSSIEKTISKAKGQPREPQVYTLPPSQEEMTKNQVSLTCLVKGFYPSDIAVEWESNGQPENNYKTTPPVLDSDGSFFLYSRLTVDKSRWQEGNVFSCSVMHEALHNHYTQKSLSLSLGGGGSGSAHPIPDSSPLLQFGGQVRQRYLYTDDACQTEAHLEIREDGTVGGAADQSPESLLQLKALKPGVIQILGVKTSRFLCQRPDGALYGSLHFDPEACSFRELLLEDGYNVYQSEAHGLPLHLPGCKSPHRDPAPRGPARFLPLPGLPPAPPEPPGILAPQPPDVGSSDPLSMVYPSQGRSPSYAS

SEQ ID NO: 31 - protein, 465 aa, synthetic construct
  REGION 1..465: note = GLP1(7-36) A8G,V16L,S18K,Y19Q,L20M,E21D,G22E,Q23E,A25V,K26R,E27L,A30E,V33K,K 34N,R36G_[19GS]_IgG4 Fc_variant [7GS]_FGF21(His29-Ser209)Q55C,N149C,G198Y
HGEGTFTSDLSKQMEEEAVRLFIEWLKNGGGGGGGGGSGGGGSGGGGSAESKYGPPCPPCPAPEFEGGPSVFLFPPKPKDTLMISRTPEVTCVVVDVSQEDPEVQFNWYVDGVEVHNAKTKPREEQFNSTYRVVSVLTVLHQDWLNGKEYKCKVSNKGLPSSIEKTISKAKGQPREPQVYTLPPSQEEMTKNQVSLTCLVKGFYPSDIAVEWESNGQPENNYKTTPPVLDSDGSFFLYSRLTVDKSRWQEGNVFSCSVMHEALHNHYTQKSLSLSLGGGGSGSAHPIPDSSPLLQFGGQVRQRYLYTDDACQTEAHLEIREDGTVGGAADQSPESLLQLKALKPGVIQILGVKTSRFLCQRPDGALYGSLHFDPEACSFRELLLEDGYNVYQSEAHGLPLHLPGCKSPHRDPAPRGPARFLPLPGLPPAPPEPPGILAPQPPDVGSSDPLSMVYPSQGRSPSYAS

SEQ ID NO: 32 - protein, 465 aa, synthetic construct
  REGION 1..465: note = GLP1(7-36) A8G,V16L,S18K,Y19Q,G22E,Q23E,A25V,K26Q,E27L,A30E,V33L,K34A,G35T,R 36G_[19GS]_IgG4 Fc_variant [7GS] FGF21(His29-Ser209)Q55C,N149C,G198Y
HGEGTFTSDLSKQLEEEAVQLFIEWLLATGGGGGGGGSGGGGSGGGGSAESKYGPPCPPCPAPEFEGGPSVFLFPPKPKDTLMISRTPEVTCVVVDVSQEDPEVQFNWYVDGVEVHNAKTKPREEQFNSTYRVVSVLTVLHQDWLNGKEYKCKVSNKGLPSSIEKTISKAKGQPREPQVYTLPPSQEEMTKNQVSLTCLVKGFYPSDIAVEWESNGQPENNYKTTPPVLDSDGSFFLYSRLTVDKSRWQEGNVFSCSVMHEALHNHYTQKSLSLSLGGGGSGSAHPIPDSSPLLQFGGQVRQRYLYTDDACQTEAHLEIREDGTVGGAADQSPESLLQLKALKPGVIQILGVKTSRFLCQRPDGALYGSLHFDPEACSFRELLLEDGYNVYQSEAHGLPLHLPGCKSPHRDPAPRGPARFLPLPGLPPAPPEPPGILAPQPPDVGSSDPLSMVYPSQGRSPSYAS

SEQ ID NO: 33 - protein, 474 aa, synthetic construct
  REGION 1..474: note = GLP1(7-36) A8G,V16L,S18K,Y19Q,G22E,Q23E,A25V,K26Q,E27L,A30E,V33L,K34A,G35T,R 36G,insPSSGEPPPE_[19GS]_IgG4 Fc_variant [7GS]_FGF21(His29-Ser209)Q55C,N149C,G198Y
HGEGTFTSDLSKQLEEEAVQLFIEWLLATGPSSGEPPPEGGGGGGGSGGGGSGGGGSAESKYGPPCPPCPAPEFEGGPSVFLFPPKPKDTLMISRTPEVTCVVVDVSQEDPEVQFNWYVDGVEVHNAKTKPREEQFNSTYRVVSVLTVLHQDWLNGKEYKCKVSNKGLPSSIEKTISKAKGQPREPQVYTLPPSQEEMTKNQVSLTCLVKGFYPSDIAVEWESNGQPENNYKTTPPVLDSDGSFFLYSRLTVDKSRWQEGNVFSCSVMHEALHNHYTQKSLSLSLGGGGSGSAHPIPDSSPLLQFGGQVRQRYLYTDDACQTEAHLEIREDGTVGGAADQSPESLLQLKALKPGVIQILGVKTSRFLCQRPDGALYGSLHFDPEACSFRELLLEDGYNVYQSEAHGLPLHLPGCKSPHRDPAPRGPARFLPLPGLPPAPPEPPGILAPQPPDVGSSDPLSMVYPSQGRSPSYAS

SEQ ID NO: 34 - protein, 474 aa, synthetic construct
  REGION 1..474: note = GLP1(7-36) insG,A8G,V16L,S18K,Y19Q,G22E,Q23E,A24R,A25V,K26Q,A30E,insPSSGAPPP S_[19GS]_IgG4 Fc_variant [7GS]_FGF21(His29-Ser209)Q55C,N149C,delP199
GHGEGTFTSDLSKQLEEERVQEFIEWLVKGRPSSGAPPPSGGGGGGGSGGGGSGGGGSAESKYGPPCPPCPAPEFEGGPSVFLFPPKPKDTLMISRTPEVTCVVVDVSQEDPEVQFNWYVDGVEVHNAKTKPREEQFNSTYRVVSVLTVLHQDWLNGKEYKCKVSNKGLPSSIEKTISKAKGQPREPQVYTLPPSQEEMTKNQVSLTCLVKGFYPSDIAVEWESNGQPENNYKTTPPVLDSDGSFFLYSRLTVDKSRWQEGNVFSCSVMHEALHNHYTQKSLSLSLGGGGSGSAHPIPDSSPLLQFGGQVRQRYLYTDDACQTEAHLEIREDGTVGGAADQSPESLLQLKALKPGVIQILGVKTSRFLCQRPDGALYGSLHFDPEACSFRELLLEDGYNVYQSEAHGLPLHLPGCKSPHRDPAPRGPARFLPLPGLPPAPPEPPGILAPQPPDVGSSDPLSMVGSQGRSPSYAS

SEQ ID NO: 35 - protein, 473 aa, synthetic construct
  REGION 1..473: note = GLP1(7-36) A8G,V16L,S18K,Y19Q,G22E,Q23E,A25V,K26Q,E27L,A30E,V33E,K34A,G35T,R 36G,insPSSGAPPPS_[19GS]_IgG4 Fc_variant [7GS]_FGF21(His29-Ser209)Q55C,N149C,delP199
HGEGTFTSDLSKQLEEEAVQLFIEWLEATGPSSGAPPPSGGGGGGGSGGGGSGGGGSAESKYGPPCPPCPAPEFEGGPSVFLFPPKPKDTLMISRTPEVTCVVVDVSQEDPEVQFNWYVDGVEVHNAKTKPREEQFNSTYRVVSVLTVLHQDWLNGKEYKCKVSNKGLPSSIEKTISKAKGQPREPQVYTLPPSQEEMTKNQVSLTCLVKGFYPSDIAVEWESNGQPENNYKTTPPVLDSDGSFFLYSRLTVDKSRWQEGNVFSCSVMHEALHNHYTQKSLSLSLGGGGSGSAHPIPDSSPLLQFGGQVRQRYLYTDDACQTEAHLEIREDGTVGGAADQSPESLLQLKALKPGVIQILGVKTSRFLCQRPDGALYGSLHFDPEACSFRELLLEDGYNVYQSEAHGLPLHLPGCKSPHRDPAPRGPARFLPLPGLPPAPPEPPGILAPQPPDVGSSDPLSMVGSQGRSPSYAS

SEQ ID NO: 36 - protein, 472 aa, synthetic construct
  REGION 1..472: note = GLP1(7-36) insG,A8G,V16L,S18I,Y19Q,G22E,Q23E,A25V,K26R,E27L,A30E,V33L,K34A,R 36G,insPKKQRLS_[19GS]_IgG4 Fc_variant [7GS]_FGF21(His29-Ser209)Q55C,N149C,delP199
GHGEGTFTSDLSIQLEEEAVRLFIEWLLAGGPKKQRLSGGGGGGGSGGGGSGGGGSAESKYGPPCPPCPAPEFEGGPSVFLFPPKPKDTLMISRTPEVTCVVVDVSQEDPEVQFNWYVDGVEVHNAKTKPREEQFNSTYRVVSVLTVLHQDWLNGKEYKCKVSNKGLPSSIEKTISKAKGQPREPQVYTLPPSQEEMTKNQVSLTCLVKGFYPSDIAVEWESNGQPENNYKTTPPVLDSDGSFFLYSRLTVDKSRWQEGNVFSCSVMHEALHNHYTQKSLSLSLGGGGSGSAHPIPDSSPLLQFGGQVRQRYLYTDDACQTEAHLEIREDGTVGGAADQSPESLLQLKALKPGVIQILGVKTSRFLCQRPDGALYGSLHFDPEACSFRELLLEDGYNVYQSEAHGLPLHLPGCKSPHRDPAPRGPARFLPLPGLPPAPPEPPGILAPQPPDVGSSDPLSMVGSQGRSPSYAS

SEQ ID NO: 37 - protein, 30 aa, synthetic construct
  REGION 1..30: note = GLP-1RA, general sequence
  SITE 10: note = misc_feature - Xaa is any amino acid, e.g., L or K
  SITE 12: note = misc_feature - Xaa is any amino acid, e.g., K or I
  SITE 14: note = misc_feature - Xaa is any amino acid, e.g., L or M
  SITE 15: note = misc_feature - Xaa is any amino acid, e.g., E or D
  SITE 18: note = misc_feature - Xaa is any amino acid, e.g., A or R
  SITE 20: note = misc_feature - Xaa is any amino acid, e.g., R or Q
  SITE 21: note = misc_feature - Xaa is any amino acid, e.g., L or E
  SITE 27: note = misc_feature - Xaa is any amino acid, e.g., L, E, K or V
  SITE 28: note = misc_feature - Xaa is any amino acid, e.g., A, N or K
  SITE 29: note = misc_feature - Xaa is any amino acid, e.g., T or G
  SITE 30: note = misc_feature - Xaa is any amino acid, e.g., G or R
HGEGTFTSDXSXQXXEEXVXXFIEWLXXXX

SEQ ID NO: 38 - protein, 9 aa, synthetic construct
  REGION 1..9: note = C-terminal peptide extension I
PSSGAPPPS

SEQ ID NO: 39 - protein, 9 aa, synthetic construct
  REGION 1..9: note = C-terminal peptide extension II
PVSGAPPPS

SEQ ID NO: 40 - protein, 10 aa, synthetic construct
  REGION 1..10: note = C-terminal peptide extension III
PSSGEPPPES

SEQ ID NO: 41 - protein, 9 aa, synthetic construct
  REGION 1..9: note = C-terminal peptide extension IV
PSSGEPPPE

SEQ ID NO: 42 - protein, 7 aa, synthetic construct
  REGION 1..7: note = C-terminal peptide extension V
PKKQRLS

SEQ ID NO: 43 - protein, 7 aa, synthetic construct
  REGION 1..7: note = C-terminal peptide extension VI
PKKIRYS

SEQ ID NO: 44 - protein, 4 aa, synthetic construct
  REGION 1..4: note = Peptide
EIRP

SEQ ID NO: 45 - protein, 6 aa, synthetic construct
  REGION 1..6: note = Peptide
TGLEAV

SEQ ID NO: 46 - protein, 6 aa, synthetic construct
  REGION 1..6: note = Peptide
TGLEAN

SEQ ID NO: 47 - protein, 181 aa, synthetic construct
  REGION 1..181: note = FGF21 variant
HPIPDSSPLLQFGGQVRQRYLYTDDAQQTEAHLEIREDGTVGGAADQSPESLLQLKALKPGVIQILGVKTSRFLCQRPDGALYGSLHFDPEACSFREEIRPDGYNVYQSEAHGLPLHLPGNKSPHRDPAPRGPARFLPLPGLPPALPEPPGILAPQPPDVGSSDPLSMVGPSQGRSPSYAS

SEQ ID NO: 48 - protein, 182 aa, synthetic construct
  REGION 1..182: note = FGF21 variant
HPIPDSSPLLQFGGQVRQRYLYTDDAQQTEAHLEIREDGTVGGAADQSPESLLQLKALKPGVIQILGVKTSRFLCQRPDGALYGSLHFDPEACSFRELLLEDGYNVYQSEAHGLPLHLPGNKSPHRDPAPRGPARFLPLPGLPPALPEPPGILAPQPPDVGSSDPLSMVTGLEAVRSPSYAS

SEQ ID NO: 49 - protein, 182 aa, synthetic construct
  REGION 1..182: note = FGF21 variant
HPIPDSSPLLQFGGQVRQRYLYTDDAQQTEAHLEIREDGTVGGAADQSPESLLQLKALKPGVIQILGVKTSRFLCQRPDGALYGSLHFDPEACSFRELLLEDGYNVYQSEAHGLPLHLPGNKSPHRDPAPRGPARFLPLPGLPPALPEPPGILAPQPPDVGSSDPLSMVTGLEANRSPSYAS

SEQ ID NO: 50 - protein, 181 aa, synthetic construct
  REGION 1..181: note = FGF21 variant
HPIPDSSPLLQFGGQVRQRYLYTDDAQQTEAHLEIREDGTVGGAADQSPESLLQLKALKPGVIQILGVKTSRFLCQRPDGALYGSLHFDPEACSFRELLLEDGYNVYQSEAHGLPLHLPGNKSPHRDPAPRGPARFLPLPGLPPALPEPPGILAPQPPDVGSSDPLSMVNPSQGRSPSYAS

SEQ ID NO: 51 - protein, 181 aa, synthetic construct
  REGION 1..181: note = FGF21 variant
HPIPDSSPLLQFGGQVRQRYLYTDDAQQTEAHLEIREDGTVGGAADQSPESLLQLKALKPGVIQILGVKTSRFLCQRPDGALYGSLHFDPEACSFRELLLEDGYNVYQSEAHGLPLHLPGNKSPHRDPAPRGPARFLPLPGLPPALPEPPGILAPQPPDVGSSDPLSMVGPSQNRSPSYAS

SEQ ID NO: 52 - protein, 182 aa, synthetic construct
  REGION 1..182: note = FGF21 variant
HPIPDSSPLLQFGGQVRQRYLYTDDAQQTEAHLEIREDGTVGGAADQSPESLLQLKALKPGVIQILGVKTSRFLCQRPDGALYGSLHFDPEACSFREEIRPDGYNVYQSEAHGLPLHLPGNKSPHRDPAPRGPARFLPLPGLPPALPEPPGILAPQPPDVGSSDPLSMVTGLEAVRSPSYAS

SEQ ID NO: 53 - protein, 182 aa, synthetic construct
  REGION 1..182: note = FGF21 variant
HPIPDSSPLLQFGGQVRQRYLYTDDAQQTEAHLEIREDGTVGGAADQSPESLLQLKALKPGVIQILGVKTSRFLCQRPDGALYGSLHFDPEACSFREEIRPDGYNVYQSEAHGLPLHLPGNKSPHRDPAPRGPARFLPLPGLPPALPEPPGILAPQPPDVGSSDPLSMVTGLEANRSPSYAS

SEQ ID NO: 54 - protein, 181 aa, synthetic construct
  REGION 1..181: note = FGF21 variant
HPIPDSSPLLQFGGQVRQRYLYTDDAQQTEAHLEIREDGTVGGAADQSPESLLQLKALKPGVIQILGVKTSRFLCQRPDGALYGSLHFDPEACSFREEIRPDGYNVYQSEAHGLPLHLPGNKSPHRDPAPRGPARFLPLPGLPPALPEPPGILAPQPPDVGSSDPLSMVNPSQGRSPSYAS

SEQ ID NO: 55 - protein, 181 aa, synthetic construct
  REGION 1..181: note = FGF21 variant
HPIPDSSPLLQFGGQVRQRYLYTDDAQQTEAHLEIREDGTVGGAADQSPESLLQLKALKPGVIQILGVKTSRFLCQRPDGALYGSLHFDPEACSFREEIRPDGYNVYQSEAHGLPLHLPGNKSPHRDPAPRGPARFLPLPGLPPALPEPPGILAPQPPDVGSSDPLSMVGPSQNRSPSYAS

SEQ ID NO: 56 - protein, 181 aa, synthetic construct
  REGION 1..181: note = FGF21 variant
HPIPDSSPLLQFGGQVRQRYLYTDDAQQTEAHLEIREDGTVGGAADQSPESLLQLKALKPGVIQILGVKTSRFLCQRPDGALYGSLHFDPEACSFREEIRPDGYNVYQSEAHGLPLHLPGNKSPHRDPAPRGPARFLPLPGLPPALPEPPGILAPQPPDVGSSDPLSMVGPSQGRSPSYES

SEQ ID NO: 57 - protein, 182 aa, synthetic construct
  REGION 1..182: note = FGF21 variant
HPIPDSSPLLQFGGQVRQRYLYTDDAQQTEAHLEIREDGTVGGAADQSPESLLQLKALKPGVIQILGVKTSRFLCQRPDGALYGSLHFDPEACSFRELLLEDGYNVYQSEAHGLPLHLPGNKSPHRDPAPRGPARFLPLPGLPPALPEPPGILAPQPPDVGSSDPLSMVTGLEAVRSPSYES

SEQ ID NO: 58 - protein, 182 aa, synthetic construct
  REGION 1..182: note = FGF21 variant
HPIPDSSPLLQFGGQVRQRYLYTDDAQQTEAHLEIREDGTVGGAADQSPESLLQLKALKPGVIQILGVKTSRFLCQRPDGALYGSLHFDPEACSFRELLLEDGYNVYQSEAHGLPLHLPGNKSPHRDPAPRGPARFLPLPGLPPALPEPPGILAPQPPDVGSSDPLSMVTGLEANRSPSYES

SEQ ID NO: 59 - protein, 181 aa, synthetic construct
  REGION 1..181: note = FGF21 variant
HPIPDSSPLLQFGGQVRQRYLYTDDAQQTEAHLEIREDGTVGGAADQSPESLLQLKALKPGVIQILGVKTSRFLCQRPDGALYGSLHFDPEACSFRELLLEDGYNVYQSEAHGLPLHLPGNKSPHRDPAPRGPARFLPLPGLPPALPEPPGILAPQPPDVGSSDPLSMVNPSQGRSPSYES

SEQ ID NO: 60 - protein, 181 aa, synthetic construct
  REGION 1..181: note = FGF21 variant
HPIPDSSPLLQFGGQVRQRYLYTDDAQQTEAHLEIREDGTVGGAADQSPESLLQLKALKPGVIQILGVKTSRFLCQRPDGALYGSLHFDPEACSFRELLLEDGYNVYQSEAHGLPLHLPGNKSPHRDPAPRGPARFLPLPGLPPALPEPPGILAPQPPDVGSSDPLSMVGPSQNRSPSYES

SEQ ID NO: 61 - protein, 182 aa, synthetic construct
  REGION 1..182: note = FGF21 variant
HPIPDSSPLLQFGGQVRQRYLYTDDAQQTEAHLEIREDGTVGGAADQSPESLLQLKALKPGVIQILGVKTSRFLCQRPDGALYGSLHFDPEACSFREEIRPDGYNVYQSEAHGLPLHLPGNKSPHRDPAPRGPARFLPLPGLPPALPEPPGILAPQPPDVGSSDPLSMVTGLEAVRSPSYES

SEQ ID NO: 62 - protein, 182 aa, synthetic construct
  REGION 1..182: note = FGF21 variant
HPIPDSSPLLQFGGQVRQRYLYTDDAQQTEAHLEIREDGTVGGAADQSPESLLQLKALKPGVIQILGVKTSRFLCQRPDGALYGSLHFDPEACSFREEIRPDGYNVYQSEAHGLPLHLPGNKSPHRDPAPRGPARFLPLPGLPPALPEPPGILAPQPPDVGSSDPLSMVTGLEANRSPSYES

SEQ ID NO: 63 - protein, 181 aa, synthetic construct
  REGION 1..181: note = FGF21 variant
HPIPDSSPLLQFGGQVRQRYLYTDDAQQTEAHLEIREDGTVGGAADQSPESLLQLKALKPGVIQILGVKTSRFLCQRPDGALYGSLHFDPEACSFREEIRPDGYNVYQSEAHGLPLHLPGNKSPHRDPAPRGPARFLPLPGLPPALPEPPGILAPQPPDVGSSDPLSMVNPSQGRSPSYES

SEQ ID NO: 64 - protein, 181 aa, synthetic construct
  REGION 1..181: note = FGF21 variant
HPIPDSSPLLQFGGQVRQRYLYTDDAQQTEAHLEIREDGTVGGAADQSPESLLQLKALKPGVIQILGVKTSRFLCQRPDGALYGSLHFDPEACSFREEIRPDGYNVYQSEAHGLPLHLPGNKSPHRDPAPRGPARFLPLPGLPPALPEPPGILAPQPPDVGSSDPLSMVGPSQNRSPSYES

SEQ ID NO: 65 - protein, 223 aa, synthetic construct
  REGION 1..223: note = Hybrid Fc variant
ETKTPECPSHTQPLGVFLFPPKPKDTLMISRTPEVTCVVVDVSQEDPEVQFNWYVDGVEVHNAKTKPREEQFNSTYRVVSVLTVLHQDWLNGKEYKCKVSNKGLPSSIEKTISKAKGQPREPQVYTLPPSQEEMTKNQVSLTCLVKGFYPSDIAVEWESNGQPENNYKTTPPVLDSDGSFFLYSRLTVDKSRWQEGNVFSCSVMHEALHNHYTQKSLSLSLGK

SEQ ID NO: 66 - protein, 245 aa, synthetic construct
  REGION 1..245: note = Hybrid Fc variant
RNTGRGGEEKKKEKEKEEQEERETKTPECPSHTQPLGVFLFPPKPKDTLMISRTPEVTCVVVDVSQEDPEVQFNWYVDGVEVHNAKTKPREEQFNSTYRVVSVLTVLHQDWLNGKEYKCKVSNKGLPSSIEKTISKAKGQPREPQVYTLPPSQEEMTKNQVSLTCLVKGFYPSDIAVEWESNGQPENNYKTTPPVLDSDGSFFLYSRLTVDKSRWQEGNVFSCSVMHEALHNHYTQKSLSLSLGK

SEQ ID NO: 67 - protein, 233 aa, synthetic construct
  REGION 1..233: note = Hybrid Fc variant
EKEKEEQEERETKTPECPSHTQPLGVFLFPPKPKDTLMISRTPEVTCVVVDVSQEDPEVQFNWYVDGVEVHNAKTKPREEQFNSTYRVVSVLTVLHQDWLNGKEYKCKVSNKGLPSSIEKTISKAKGQPREPQVYTLPPSQEEMTKNQVSLTCLVKGFYPSDIAVEWESNGQPENNYKTTPPVLDSDGSFFLYSRLTVDKSRWQEGNVFSCSVMHEALHNHYTQKSLSLSLGK

SEQ ID NO: 68 - protein, 255 aa, synthetic construct
  REGION 1..255: note = Hybrid Fc variant
AKATTAPATTRNTGRGGEEKKKEKEKEEQEERETKTPECPSHTQPLGVFLFPPKPKDTLMISRTPEVTCVVVDVSQEDPEVQFNWYVDGVEVHNAKTKPREEQFNSTYRVVSVLTVLHQDWLNGKEYKCKVSNKGLPSSIEKTISKAKGQPREPQVYTLPPSQEEMTKNQVSLTCLVKGFYPSDIAVEWESNGQPENNYKTTPPVLDSDGSFFLYSRLTVDKSRWQEGNVFSCSVMHEALHNHYTQKSLSLSLGK

SEQ ID NO: 69 - protein, 264 aa, synthetic construct
  REGION 1..264: note = Hybrid Fc variant
AQPQAEGSLAKATTAPATTRNTGRGGEEKKKEKEKEEQEERETKTPECPSHTQPLGVFLFPPKPKDTLMISRTPEVTCVVVDVSQEDPEVQFNWYVDGVEVHNAKTKPREEQFNSTYRVVSVLTVLHQDWLNGKEYKCKVSNKGLPSSIEKTISKAKGQPREPQVYTLPPSQEEMTKNQVSLTCLVKGFYPSDIAVEWESNGQPENNYKTTPPVLDSDGSFFLYSRLTVDKSRWQEGNVFSCSVMHEALHNHYTQKSLSLSLGK

SEQ ID NO: 70 - protein, 253 aa, synthetic construct
  REGION 1..253: note = Hybrid Fc variant
ETKTPECPSHTQPLGVFLFPPKPKDTLMISRTPEVTCVVVDVSQEDPEVQFNWYVDGVEVHNAKTKPREEQFNSTYRVVSVLTVLHQDWLNGKEYKCKVSNKGLPSSIEKTISKAKGQPREPQVYTLPPSQEEMTKNQVSLTCLVKGFYPSDIAVEWESNGQPENNYKTTPPVLDSDGSFFLYSRLTVDKSRWQEGNVFSCSVMHEALHNHYTQKSLSLSLGKAKATTAPATTRNTGRGGEEKKKEKEKEEQE